European Patent Specification EP 3 430 041 B1, published May 24, 2023. Title: Anti-TNF-alpha antibodies and functional fragments thereof. Applicant: Numab Innovation AG. The sequence listing filed with the application follows.

SEQUENCE LISTING (44 sequences)

SEQ ID NO: 1 - protein, 11 aa, Artificial Sequence
  Generic CDR L1
  MISC_FEATURE (4)..(4): Xaa is Glu or Gln
  MISC_FEATURE (5)..(5): Xaa is Ser or Asn
  MISC_FEATURE (7)..(7): Xaa is Gly or Tyr
  MISC_FEATURE (8)..(8): Xaa is Asn or Ser
  MISC_FEATURE (9)..(9): Xaa is Ala or Asp
QASXXIXXXLA

SEQ ID NO: 2 - protein, 7 aa, Artificial Sequence
  Generic CDR L2
  MISC_FEATURE (1)..(1): Xaa is Ser, Gly or Gln
  MISC_FEATURE (4)..(4): Xaa is Thr or Lys
XASXLAS

SEQ ID NO: 3 - protein, 13 aa, Artificial Sequence
  Generic CDR L3
  MISC_FEATURE (11)..(11): Xaa os Tyr or Asp
QSYYYSSSGSXVA

SEQ ID NO: 4 - protein, 11 aa, Artificial Sequence
  Generic CDR H1
  MISC_FEATURE (5)..(5): Xaa is Asn or Ser
  MISC_FEATURE (6)..(6): Xaa is Asn or Lys
  MISC_FEATURE (10)..(10): Xaa is Met, Ile or Ala
GIDFXXYYFXC

SEQ ID NO: 5 - protein, 17 aa, Artificial Sequence
  Generic CDR H2
  MISC_FEATURE (6)..(6): Xaa is Ser or Thr
  MISC_FEATURE (7)..(7): Xaa is Asp or Gly
  MISC_FEATURE (9)..(9): Xaa is Thr or Ile
  MISC_FEATURE (11)..(11): Xaa is Tyr or Phe
  MISC_FEATURE (13)..(13): Xaa is Ser or Thr
CINTGXXSXYXAXWAKG

SEQ ID NO: 6 - protein, 16 aa, Artificial Sequence
  Generic CDR H3
  MISC_FEATURE (8)..(8): Xaa is Val or Tyr
  MISC_FEATURE (15)..(15): Xaa is Ser or His
ASGSSSVXYIGVYFXL

SEQ ID NO: 7 - protein, 11 aa, Artificial Sequence
  CDR L1 of clone 16-12-C02 and clone 17-21-A01
QASESIGNALA

SEQ ID NO: 8 - protein, 11 aa, Artificial Sequence
  CDR L1 of clone 16-14-C04, clone 16-14-G10, clone 16-17-E05 and clone 16-19-G09
QASQNIYSDLA

SEQ ID NO: 9 - protein, 7 aa, Artificial Sequence
  CDR L2 of 16-12-C02 and clone 17-21-A01
SASTLAS

SEQ ID NO: 10 - protein, 7 aa, Artificial Sequence
  CDR L2 of clone 16-14-C04 and clone 16-14-G10
GASTLAS

SEQ ID NO: 11 - protein, 7 aa, Artificial Sequence
  CDR L2 of clone 16-17-E05 and clone 16-19-G09
QASKLAS

SEQ ID NO: 12 - protein, 13 aa, Artificial Sequence
  CDR L3 of clone 16-12-C02 and clone 17-21-A01
QSYYYSSSGSYVA

SEQ ID NO: 13 - protein, 13 aa, Artificial Sequence
  CDR L3 of clone 16-14-C04, clone 16-14-G10, clone 16-17-E05 and clone 16-19-G09
QSYYYSSSGSDVA

SEQ ID NO: 14 - protein, 11 aa, Artificial Sequence
  CDR H1 of clone 16-12-C02 and clone 17-21-A01
GIDFNKYYFMC

SEQ ID NO: 15 - protein, 11 aa, Artificial Sequence
  CDR H1 of clone 16-14-C04
GIDFNNYYFIC

SEQ ID NO: 16 - protein, 11 aa, Artificial Sequence
  CDR H1 of clone 16-14-G10
GIDFNKYYFIC

SEQ ID NO: 17 - protein, 11 aa, Artificial Sequence
  CDR H1 of clone 16-17-E05
GIDFSNYYFAC

SEQ ID NO: 18 - protein, 11 aa, Artificial Sequence
  CDR H1 of clone 16-19-G09
GIDFSNYYFIC

SEQ ID NO: 19 - protein, 17 aa, Artificial Sequence
  CDR H2 of clone 16-12-C02
CINTGSDSTYYASWAKG

SEQ ID NO: 20 - protein, 17 aa, Artificial Sequence
  CDR H2 of clone 16-14-C04
CINTGTGSTYYASWAKG

SEQ ID NO: 21 - protein, 17 aa, Artificial Sequence
  CDR H2 of clone 16-14-G10
CINTGTGSTYFASWAKG

SEQ ID NO: 22 - protein, 17 aa, Artificial Sequence
  CDR H2 of clone 16-17-E05
CINTGSGSIYYASWAKG

SEQ ID NO: 23 - protein, 17 aa, Artificial Sequence
  CDR H2 of clone 16-19-G09
CINTGSGSTYYASWAKG

SEQ ID NO: 24 - protein, 17 aa, Artificial Sequence
  CDR H2 of clone 17-21-A01
CINTGSGSTYYATWAKG

SEQ ID NO: 25 - protein, 16 aa, Artificial Sequence
  CDR H3 of clone 16-12-C02 and clone 17-21-A01
ASGSSSVVYIGVYFSL

SEQ ID NO: 26 - protein, 16 aa, Artificial Sequence
  CDR H3 of clone 16-14-C04, clone 16-14-G10, clone 16-17-E05 and clone 16-19-G09
ASGSSSVYYIGVYFHL

SEQ ID NO: 27 - protein, 112 aa, Artificial Sequence
  VL of humanized scFv of clone 17-21-A01-sc01
DIQMTQSPSSLSASVGDRVTITCQASESIGNALAWYQQKPGKAPKLLIYSASTLASGVPSRFSGSGSGTDFTLTISSLQPEDFATYYCQSYYYSSSGSYVAFGGGTKLTVLG

SEQ ID NO: 28 - protein, 126 aa, Artificial Sequence
  VH of humanized scFv of clone 17-21-A01-sc01
EVQLVESGGGLVQPGGSLRLSCAASGIDFNKYYFMCWVRQAPGKGLEWIGCINTGSGSTYYATWAKGRFTISRDNSKNTVYLQMNSLRAEDTAVYYCARASGSSSVVYIGVYFSLWGQGTLVTVSS

SEQ ID NO: 29 - protein, 259 aa, Artificial Sequence
  Humanized scFv of clone 17-21-A01-sc01
MDIQMTQSPSSLSASVGDRVTITCQASESIGNALAWYQQKPGKAPKLLIYSASTLASGVPSRFSGSGSGTDFTLTISSLQPEDFATYYCQSYYYSSSGSYVAFGGGTKLTVLGGGGGSGGGGSGGGGSGGGGSEVQLVESGGGLVQPGGSLRLSCAASGIDFNKYYFMCWVRQAPGKGLEWIGCINTGSGSTYYATWAKGRFTISRDNSKNTVYLQMNSLRAEDTAVYYCARASGSSSVVYIGVYFSLWGQGTLVTVSS

SEQ ID NO: 30 - protein, 112 aa, Artificial Sequence
  VL of humanized scFv of clone 17-21-A01-sc02
DIQMTQSPSSLSASVGDRVTIKCQASESIGNALAWYQQKPGKAPKLLIYSASTLASGVPSRFSGSGSGTEFTLTISDLEPADFATYYCQSYYYSSSGSYVAFGGGTKLTVLG

SEQ ID NO: 31 - protein, 126 aa, Artificial Sequence
  VH of humanized scFv of clone 17-21-A01-sc02
EVQLVESGGGLVQPGGSLRLSCKASGIDFNKYYFMCWVRQAPGKGLEWIGCINTGSGSTYYATWAKGRFTISKDSSKNTVYLQMNSLRAEDTAVYYCARASGSSSVVYIGVYFSLWGQGTLVTVSS

SEQ ID NO: 32 - protein, 259 aa, Artificial Sequence
  Humanized scFv of clone 17-21-A01-sc02
MDIQMTQSPSSLSASVGDRVTIKCQASESIGNALAWYQQKPGKAPKLLIYSASTLASGVPSRFSGSGSGTEFTLTISDLEPADFATYYCQSYYYSSSGSYVAFGGGTKLTVLGGGGGSGGGGSGGGGSGGGGSEVQLVESGGGLVQPGGSLRLSCKASGIDFNKYYFMCWVRQAPGKGLEWIGCINTGSGSTYYATWAKGRFTISKDSSKNTVYLQMNSLRAEDTAVYYCARASGSSSVVYIGVYFSLWGQGTLVTVSS

SEQ ID NO: 33 - protein, 112 aa, Artificial Sequence
  VL of humanized scFv of clone 17-21-A01-sc03
DIQMTQSPSSLSASVGDRVTITCQASESIGNALAWYQQKPGKAPKLLIYSASTLASGVPSRFSGSGSGTDFTLTISSLQPEDFATYYCQSYYYSSSGSYVAFGCGTKLTVLG

SEQ ID NO: 34 - protein, 126 aa, Artificial Sequence
  VH of humanized scFv of clone 17-21-A01-sc03
EVQLVESGGGLVQPGGSLRLSCAASGIDFNKYYFMCWVRQAPGKCLEWIGCINTGSGSTYYATWAKGRFTISRDNSKNTVYLQMNSLRAEDTAVYYCARASGSSSVVYIGVYFSLWGQGTLVTVSS

SEQ ID NO: 35 - protein, 259 aa, Artificial Sequence
  Humanized scFv of clone 17-21-A01-sc03
MDIQMTQSPSSLSASVGDRVTITCQASESIGNALAWYQQKPGKAPKLLIYSASTLASGVPSRFSGSGSGTDFTLTISSLQPEDFATYYCQSYYYSSSGSYVAFGCGTKLTVLGGGGGSGGGGSGGGGSGGGGSEVQLVESGGGLVQPGGSLRLSCAASGIDFNKYYFMCWVRQAPGKCLEWIGCINTGSGSTYYATWAKGRFTISRDNSKNTVYLQMNSLRAEDTAVYYCARASGSSSVVYIGVYFSLWGQGTLVTVSS

SEQ ID NO: 36 - protein, 20 aa, Artificial Sequence
  Linker sequence in scFv
GGGGSGGGGSGGGGSGGGGS

SEQ ID NO: 37 - protein, 5 aa, Artificial Sequence
  Linker sequence in diabody
GGGGS

SEQ ID NO: 38 - protein, 23 aa, Artificial Sequence
  Vk1 consensus sequence of framework I (Kabat positions 1-23)
DIQMTQSPSSLSASVGDRVTITC

SEQ ID NO: 39 - protein, 15 aa, Artificial Sequence
  Vk1 consensus sequence of framework II (Kabat positions 35-49)
WYQQKPGKAPKLLIY

SEQ ID NO: 40 - protein, 32 aa, Artificial Sequence
  Vk1 consensus sequence of framework III (Kabat positions 57-88)
GVPSRFSGSGSGTDFTLTISSLQPEDFATYYC

SEQ ID NO: 41 - protein, 10 aa, Artificial Sequence
  V lamda germline-based sequence of framework IV
FGTGTKVTVL

SEQ ID NO: 42 - protein, 10 aa, Artificial Sequence
  V lamda germline-based sequence of framework IV
FGGGTKLTVL

SEQ ID NO: 43 - protein, 10 aa, Artificial Sequence
  V lamda germline-based sequence of framework IV
FGGGTQLIIL

SEQ ID NO: 44 - protein, 10 aa, Artificial Sequence
  V lamda germline-based sequence of framework IV
FGSGTKVTVL